European Patent Application EP 4 163 379 A1, published April 12, 2023. Title: METHOD FOR IDENTIFYING AND/OR REGULATING SENESCENCE. Applicant: INSTITUTE OF ZOOLOGY, CHINESE ACADEMY OF SCIENCES BEIJING INSTITUTE FOR STEM CELL AND REGENERATIVE MEDICINE. The sequence listing filed with the application follows.

SEQUENCE LISTING (153 sequences)

SEQ ID NO: 1 - protein, 560 aa, Homo sapiens
MVTPVTWMDNPIEVYVNDSVWVPGPTDDRCPAKPEEEGMMINISIGYHYPPICLGRAPGCLMPAVQNWLVEVPTVSPNSRFTYHMVSGMSLRPRVNCLQDFSYQRSLKFRPKGKTCPKEIPKGSKNTEVLVWEECVANSVVILQNNEFGTIIDWAPRGQFYHNCSGQTQSCPSAQVSPAVDSDLTESLDKHKHKKLQSFYLWEWEEKGISTPRPKIISPVSGPEHPELWRLTVASHHIRIWSGNQTLETRYRKPFYTIDLNSILTVPLQSCVKPPYMLVVGNIVIKPASQTITCENCRLFTCIDSTFNWQHRILLVRAREGMWIPVSTDRPWEASPSIHILTEILKGVLNRSKRFIFTLIAVIMGLIAVTATAAVAGVALHSSVQSVNFVNYWQKNSTRLWNSQSSIDQKLASQINDLRQTVIWMGDRLMTLEHHFQLQCDWNTSDFCITPQIYNESEHHWDMVRRHLQGREDNLTLDISKLKEQIFEASKAHLNLVPGTEAIAGVADGLANLNPVTWIKTIRSTMIINLILIVVCLFCLLLVCRCTQQLRRDSDIENGP

SEQ ID NO: 2 - protein, 702 aa, Homo sapiens
MIPKDWPLIIIDLKDCFFTIPLAEQDCEKFAFTIPAINNKEPATRFQWKVLPQGMLNSPTLCQTFVGRALQPVRDKFSDCYIIHYFDDILCAAETKDKLIDCYTFLQAEVANAGLAIASDKIQTSTPFHYLGMQIENRKIKPQKIEIRKDTLKTLNDFQKLLGDINWIRPTLGIPTYAMSNLFSILRGDSDLNSKRMLTPEATKEIKLVEEKIQSAQINRIDPLAPLQLLIFATAHSPTGIIIQNTDLVEWSFLPHSTVKTFTLYLDQIATLIGPTRLRIIKLCGNDPDKIVVPLTKEQVRQAFINSGAWQIGLANFVGIIDNHYPKTKIFQFLKLTTWILPKITRREPLENALTVFTDGSSNGKVAYTGPKERVIKTPYQSAQRAELVAVITVLQDFDQPINIISDSAYVVQATRDVETALIKYSMDDQLNQLFNLLQQTVRKRNFPFYITHIRAHTNLPGPLTKANEQADLLVSSAFIKAQELHALTHVNAAGLKNKFDVTWKQAKDIVQHCTQCQVLDLPTQEAGVNPEVCVLMHYGKWMSHMYLHLGRLSYVHVTVDTYSHFMCATCQTGESTSHVKKHLLSCFAVMGVPEKIKTDNGPGYCSKAFQKFLSQWKISHTTGIPYNSQGQAIVERTNRTLKTQLVKQKEGGDSKECTTPQMQLNLALYTLNFLNIYRNQTTTSAEHLTGKKNSPHEGKLI

SEQ ID NO: 3 - protein, 334 aa, Homo sapiens
KWATIVGKRAKGPASGPTTNWGIPNSAICSSGFSGTTTPTVPSVSGNKPVTTIQQLSPATSGSAAVDLCTIQAVSLLPGEPPQKIPTGVYGPLPEGTVGLILGRSSLNLKGVQIHTSVVDSDYKGEIQLVISSSIPWSASPGDRIAQLLLLPYIKGGNSEIKRIGGLGSTDPTGKAAYWASQVSENRPVCKAIIQGKQFEGLVDTGADVSIIALNQWPKNWPKQKAVTGLVGIGTASEVYQSTEILHCLGPDNQESTVQPMITSIPLNLWGRDLLQQWGAEITMPAPLYSPTSQKIMTKMGYIPGKGLGKNEDGIKIPVEAKINQKREGIGYPF

SEQ ID NO: 4 - protein, 253 aa, Homo sapiens
MGQTKTKSKYASYLSFIKILLKRGGVRVSTKNLIKLFQTTEQFCPWFPEQGNLDLEDWKRIGKELKQAGRKGNIIPLTVWNDWPIIKAALEPFQTEDSVSVSDAPGSCIIDCNEKTRKKSQKETETLHCEYVAEPLMAQSTQNVDYNQLQEVIYPETLKLEGKGPELVGPLESKPRGPSPLSAGQVTVTLQPQAQVRENKTQLPVAYQYWPPAELQYRPPPESQYGYLGMPPAPQDREPYPQPPTRRQCYGTT

SEQ ID NO: 5 - DNA, 1683 bp, Homo sapiens
atggtaacaccagtcacatggatggataatcctatagaagtatatgttaatgatagtgtatgggtacctggccccacagatgatcgctgccctgccaaacctgaggaagaagggatgatgataaatatttccattgggtatcattatcctcctatttgcctagggagagcaccaggatgtttaatgcctgcagtccaaaattggttggtagaagtacctactgtcagtcctaacagtagattcacttatcacatggtaagcgggatgtcactcaggccacgggtaaattgtttacaagacttttcttatcaaagatcattaaaatttagacctaaagggaaaacttgccccaaggaaattcctaaaggatcaaagaatacagaagttttagtttgggaagaatgtgtggccaatagtgtggtgatattacaaaacaatgaattcggaactattatagattgggcacctcgaggtcaattctaccacaattgctcaggacaaactcagtcgtgtccaagtgcacaagtgagtccagctgtcgatagcgacttaacagaaagtctagacaaacataagcataaaaaattacagtctttctacctttgggaatgggaagaaaaaggaatctctaccccaagaccaaaaataataagtcctgtttctggtcctgaacatccagaattgtggaggcttactgtggcctcacaccacattagaatttggtctggaaatcaaactttagaaacaagatatcgtaagccattttatactatcgacctaaattccattctaacggttcctttacaaagttgcgtaaagcccccttatatgctagttgtaggaaatatagttattaaaccagcctcccaaactataacctgtgaaaattgtagattgtttacttgcattgattcaacttttaattggcagcaccgtattctgctggtgagagcaagagaaggcatgtggatccctgtgtccacggaccgaccgtgggaggcctcgccatccatccatattttgactgaaatattaaaaggcgttttaaatagatccaaaagattcatttttactttaattgcagtgattatgggattaattgcagtcacagctacggctgctgtggcaggagttgcattgcactcttctgttcagtcagtaaactttgttaattattggcaaaagaattctacaagattgtggaattcacaatctagtattgatcaaaaattggcaagtcaaattaatgatcttagacaaactgtcatttggatgggagacaggctcatgaccttagaacatcatttccagttacagtgtgactggaatacgtcagatttttgtattacaccccaaatttataatgagtctgagcatcactgggacatggttagacgccatctacagggaagagaagataatctcactttagacatttccaaattaaaagaacaaattttcgaagcatcaaaagcccatttaaatttggtgccaggaactgaggcaattgcaggagttgctgatggcctcgcaaatcttaaccctgtcacttggattaagaccatcagaagtactatgattataaatctcatattaatcgttgtgtgcctgttttgtctgttgttagtctgcaggtgtacccaacagctccgaagagacagtgacatcgagaacgggccatga

SEQ ID NO: 6 - DNA, 2109 bp, Homo sapiens
atgatcccaaaagattggcctttaattataattgatctaaaggactgcttttttaccatccctctggcagagcaggattgtgaaaaatttgcctttactataccagccataaataataaagaaccagccaccaggtttcagtggaaagtgttacctcagggaatgcttaatagtccaactctttgtcagacttttgtaggtcgagctcttcaaccagttagagacaagttttcagactgttatattattcattattttgatgatattttatgtgctgcagaaacgaaagataaattaattgactgttatacatttctgcaagcagaggttgccaatgcaggactggcaatagcatctgataagatccaaacctctactccttttcattatttagggatgcagatagaaaatagaaaaattaagccacaaaaaatagaaataagaaaagacacattaaaaacactaaatgattttcaaaaattgctgggagatattaattggattcggccaactctaggcattcctacttatgccatgtcaaatttgttctctatcttaagaggagactcagacttaaatagtaaaagaatgttaaccccagaggcaacaaaagaaattaaattagtggaagaaaaaattcagtcagcgcaaataaatagaatagatcccttagccccactccaacttttgatttttgccactgcccattctccaacaggcatcattattcaaaatactgatcttgtggagtggtcattccttcctcacagtacagttaagacttttacattgtacttggatcaaatagctactttaattggtccgacaagattacgaataataaaattatgtggaaatgacccagacaaaatagttgtccctttaaccaaggaacaagttagacaagcctttatcaattctggtgcatggcagattggtcttgctaattttgtgggaattattgataatcattacccaaaaacaaaaatcttccagttcttaaaattgactacttggattctacctaaaattaccagacgtgaacctttagaaaatgctctaacagtatttactgatggttccagcaatggaaaagtggcttacacagggccaaaagaacgagtaatcaaaactccatatcaatcggctcaaagagcagagttggttgcagtcattacagtgttacaagattttgatcaacctatcaatattatatcggattctgcatatgtagtacaggctacaagggatgttgagacagctctaattaaatatagcatggacgatcagttaaaccagctattcaatttattacaacaaactgtaagaaaaagaaacttcccattttatattactcatattcgagcacacactaatttaccagggcctttgactaaagcaaatgaacaagctgacttactggtatcatctgcattcataaaagcacaagaacttcatgctttgactcatgtaaatgcagcaggattaaaaaacaaatttgatgtcacatggaaacaggcaaaagatattgtacaacattgcacccagtgtcaagtcttagacctgcccactcaagaggcaggagttaacccagaggtctgtgtcctaatgcattatggcaaatggatgtcacacatgtaccttcatttgggaagattatcatatgttcatgtaacagttgatacttattcacatttcatgtgtgcaacttgccaaacaggagaaagtacttcccatgttaaaaaacatttattgtcttgttttgctgtaatgggagttccagaaaaaatcaaaactgacaatggaccaggatattgtagtaaagctttccaaaaattcttaagtcagtggaaaatttcacatacaacaggaattccttataattcccaaggacaggccatagttgaaagaactaatagaacactcaaaactcaattagttaaacaaaaagaagggggagacagtaaggagtgtaccactcctcagatgcaacttaatctagcactctatactttaaattttttaaacatttatagaaatcagactactacttctgcagaacatcttactggtaaaaagaacagcccacatgaaggaaaactaatttag

SEQ ID NO: 7 - DNA, 1005 bp, Homo sapiens
aatgggcaaccattgtcgggaaacgagcaaaggggccagcctcaggccccacaacaaactggggcattcccaattcagccatttgttcctcagggttttcagggacaacaacccccactgtcccaagtgtttcagggaataagccagttaccacaatacaacaattgtcccccgccacaagcggcagtgcagcagtagatttatgtactatacaagcagtctctctgcttccaggggagcccccacaaaaaatccccacaggggtatatggccccctgcctgaggggactgtaggactaatcttgggaagatcaagtctaaatctaaaaggagttcaaattcatactagtgtggttgattcagactataaaggcgaaattcaattggttattagctcttcaattccttggagtgccagtccaggagacaggattgctcaattattactcctgccatatattaagggtggaaatagtgaaataaaaagaataggagggcttggaagcactgatccaacaggaaaggctgcatattgggcaagtcaggtctcagagaacagacctgtgtgtaaggccattattcaaggaaaacagtttgaagggttggtagacactggagcagatgtctctatcattgctttaaatcagtggccaaaaaattggcctaaacaaaaggctgttacaggacttgtcggcataggcacagcctcagaagtgtatcaaagtacggagattttacattgcttagggccagataatcaagaaagtactgttcagccaatgattacttcaattcctcttaatctgtggggtcgagatttattacaacaatggggtgcggaaatcaccatgcccgctccattatatagccccacgagtcaaaaaatcatgaccaagatgggatatataccaggaaagggactagggaaaaatgaagatggcattaaaattccagttgaggctaaaataaatcaaaaaagagaaggaatagggtatcctttttagg

SEQ ID NO: 8 - DNA, 762 bp, Homo sapiens
atggggcaaactaaaactaaaagtaaatatgcctcttatcttagcttcattaaaattcttttaaaaagagggggagttagagtatccaccaaaaatctaatcaagctatttcaaacaacagaacaattttgcccatggtttccagaacaaggaaatttagatctagaagattggaaaagaattggtaaggaactaaaacaagcaggtaggaagggtaatatcattccacttacagtatggaatgattggcccattattaaagcagctttagaaccatttcaaacagaagatagcgtttcagtttctgatgcccctggaagctgtataatagattgtaatgaaaagacaaggaaaaaatcccagaaggaaacggaaactttacattgcgaatatgtagcagagccgttaatggctcagtcaacgcaaaatgttgactataatcaattacaggaggtgatatatcctgaaacattaaaattagaaggaaaaggtccagaattagtggggccattagagtctaaaccacgagggccaagtcctctttcagcaggtcaggtgaccgtaacattacaacctcaagcgcaggttagagaaaataagacccaactgccagtagcttatcaatactggccaccggccgaacttcagtatcggccacccccagaaagtcagtatggatatctaggaatgccaccagcaccacaggacagggagccataccctcagccgcccactaggagacaatgctatggcaccacctag

SEQ ID NO: 9 - DNA, 20 bp, Artificial Sequence
  primer
gggcagcaatactgctttgt

SEQ ID NO: 10 - DNA, 20 bp, Artificial Sequence
  primer
caatagtggggagagggtca

SEQ ID NO: 11 - DNA, 18 bp, Artificial Sequence
  primer
tcgaagcatcaaaagccc

SEQ ID NO: 12 - DNA, 22 bp, Artificial Sequence
  primer
gcagactaacaacagacaaaac

SEQ ID NO: 13 - DNA, 21 bp, Artificial Sequence
  primer
ccagcctcccaaactataacc

SEQ ID NO: 14 - DNA, 19 bp, Artificial Sequence
  primer
aagagtgcaatgcaactcc

SEQ ID NO: 15 - DNA, 24 bp, Artificial Sequence
  primer
aaataagacccaaccgccagtagc

SEQ ID NO: 16 - DNA, 24 bp, Artificial Sequence
  primer
gaattgccatgcctcagtatctcc

SEQ ID NO: 17 - DNA, 19 bp, Artificial Sequence
  primer
cccagaaggaaacggaaac

SEQ ID NO: 18 - DNA, 19 bp, Artificial Sequence
  primer
tgacctgctgaaagaggac

SEQ ID NO: 19 - DNA, 22 bp, Artificial Sequence
  primer
gccgatgaaaaagcccgtaagg

SEQ ID NO: 20 - DNA, 24 bp, Artificial Sequence
  primer
ttgacactcaggattggcgttttc

SEQ ID NO: 21 - DNA, 20 bp, Artificial Sequence
  primer
tttgccactgcccattctcc

SEQ ID NO: 22 - DNA, 20 bp, Artificial Sequence
  primer
aagaccaatctgccatgcac

SEQ ID NO: 23 - DNA, 20 bp, Artificial Sequence
  primer
tcatgatgatgggcagcgcc

SEQ ID NO: 24 - DNA, 20 bp, Artificial Sequence
  primer
acgggtcgggtgagagtggc

SEQ ID NO: 25 - DNA, 19 bp, Artificial Sequence
  primer
tgtccgtcagaacccatgc

SEQ ID NO: 26 - DNA, 21 bp, Artificial Sequence
  primer
aaagtcgaagttccatcgctc

SEQ ID NO: 27 - DNA, 23 bp, Artificial Sequence
  primer
accagaaggaagcatgaaacgcg

SEQ ID NO: 28 - DNA, 23 bp, Artificial Sequence
  primer
tcatctcatgaagggcctgagcc

SEQ ID NO: 29 - DNA, 20 bp, Artificial Sequence
  primer
cccctcggtcctgacaaaag

SEQ ID NO: 30 - DNA, 20 bp, Artificial Sequence
  primer
cgctcttcgtcactggagaa

SEQ ID NO: 31 - DNA, 20 bp, Artificial Sequence
  primer
acgccgcattgaccatctat

SEQ ID NO: 32 - DNA, 20 bp, Artificial Sequence
  primer
gtctcattccagccagtgct

SEQ ID NO: 33 - DNA, 22 bp, Artificial Sequence
  primer
cgccagtgaaatgatggcttat

SEQ ID NO: 34 - DNA, 22 bp, Artificial Sequence
  primer
ctggaaggagcacttcatctgt

SEQ ID NO: 35 - DNA, 23 bp, Artificial Sequence
  primer
actgacctcttcagaacgaattg

SEQ ID NO: 36 - DNA, 23 bp, Artificial Sequence
  primer
ccatctttggaaggttcaggttg

SEQ ID NO: 37 - DNA, 23 bp, Artificial Sequence
  primer
actgagagtgattgagagtggac

SEQ ID NO: 38 - DNA, 21 bp, Artificial Sequence
  primer
aaccctctgcacccatggttc

SEQ ID NO: 39 - DNA, 20 bp, Artificial Sequence
  primer
agagctacgagctgcctgac

SEQ ID NO: 40 - DNA, 20 bp, Artificial Sequence
  primer
agcactgtgttggcgtacag

SEQ ID NO: 41 - DNA, 20 bp, Artificial Sequence
  primer
tcggagtcaacggatttggt

SEQ ID NO: 42 - DNA, 20 bp, Artificial Sequence
  primer
ttgccatgggtggaatcata

SEQ ID NO: 43 - DNA, 23 bp, Artificial Sequence
  primer
ctcgtctgatctcggaagctaag

SEQ ID NO: 44 - DNA, 20 bp, Artificial Sequence
  primer
gcggtctcccatccaagtac

SEQ ID NO: 45 - DNA, 20 bp, Artificial Sequence
  primer
ggagagaagctgtcctgtgg

SEQ ID NO: 46 - DNA, 20 bp, Artificial Sequence
  primer
tgactggacttgcacgtagg

SEQ ID NO: 47 - DNA, 20 bp, Artificial Sequence
  primer
gatggtatgaagcaggatgg

SEQ ID NO: 48 - DNA, 34 bp, Artificial Sequence
  primer
cctcttttctctatatctattagctgaggtaatc

SEQ ID NO: 49 - DNA, 20 bp, Artificial Sequence
  primer
gatggtatgaagcaggatgg

SEQ ID NO: 50 - DNA, 26 bp, Artificial Sequence
  primer
aagggtaagtaacacaggcagatgta

SEQ ID NO: 51 - DNA, 19 bp, Artificial Sequence
  shRNA
cctgaacatccagaattat

SEQ ID NO: 52 - DNA, 20 bp, Artificial Sequence
  shRNA
acattattagattccattgc

SEQ ID NO: 53 - DNA, 21 bp, Artificial Sequence
  shRNA
gcccggattcgaacttacaat

SEQ ID NO: 54 - DNA, 20 bp, Artificial Sequence
  sgRNA
acggaggctaagcgtcgcaa

SEQ ID NO: 55 - DNA, 20 bp, Artificial Sequence
  sgRNA
acgggcggctatcgctgact

SEQ ID NO: 56 - DNA, 20 bp, Artificial Sequence
  sgRNA
tctctcatttgaacatccac

SEQ ID NO: 57 - DNA, 20 bp, Artificial Sequence
  sgRNA
aagatgaaaggaaaggcgtt

SEQ ID NO: 58 - DNA, 20 bp, Artificial Sequence
  sgRNA
ctgaaaaaggaaggagttga

SEQ ID NO: 59 - DNA, 23 bp, Artificial Sequence
  sgRNA
gatagggaaaaaccgccttaggg

SEQ ID NO: 60 - DNA, 1054 bp, Artificial Sequence
  probe
cggcagtgcagcaagtagatttatgtactatacaagcagtctctctgcttccaggggagcccccacaaaaaacccccacaggggtatatggacccctgcctaaggggactgtaggactaatcttgggacgatcaagtctaaatctaaaaggagttcaaattcatactagtgtggttgattcagactataaaggcgaaattcaattggttattagctcttcaattccttggagtgccagtccaagagacaggattgctcaattattactcctgccatacattaagggtggaaatagtgaaataaaaagaataggagggcttggaagcactgatccaacaggaaaggctgcatattgggcaagtcaggtctcagagaacagacctgtgtgtaaggccattattcaaggaaaacagtttgaagggttggtagacactggagcagatgtctctatcattgctttaaatcagtggccaaaaaattggcctaaacaaaaggctgttacaggacttgtcggcataggcacagcctcagaagtgtatcaaagtacggagattttacattgcttagggccagataatcaagaaagtactgttcagccaatgattacttcaattcctcttaatctgtggggtcgagatttattacaacaatggggtgcggaaatcaccatgcccgctccatcatatagccccacgagtcaaaaaatcatgaccaagatgggatatataccaggaaagggactagggaaaaatgaagatggcattaaaattccagttgaggctaaaataaatcaagaaagagaaggaatagggaatccttgcctaggggcggccactgtagagcctcctaaacccataccattaacttggaaaacagaaaaaccagtgtgggtaaatcagtggccgctaccaaaacaaaaactggaggctttacatttattagcaaatgaacagttagaaaagggtcatattgagccttcgttctcaccttggaattctcctgtgtttgtaattcagaagaaatcaggcaaatggcgtatgttaactgacttaag

SEQ ID NO: 61 - DNA, 21 bp, Artificial Sequence
  sgRNA
accccgtgctctctgaaacac

SEQ ID NO: 62 - DNA, 23 bp, Artificial Sequence
  sgRNA
tgtgaaccttgcggttcccaagg

SEQ ID NO: 63 - DNA, 25 bp, Artificial Sequence
  probe
ctaatcaagctatttcaaacaacag

SEQ ID NO: 64 - DNA, 25 bp, Artificial Sequence
  probe
acaattttgcccatggtttccagaa

SEQ ID NO: 65 - DNA, 25 bp, Artificial Sequence
  probe
atttagatctagaagattggaaaag

SEQ ID NO: 66 - DNA, 25 bp, Artificial Sequence
  probe
attggtaaggaactaaaacaagcag

SEQ ID NO: 67 - DNA, 25 bp, Artificial Sequence
  probe
tccacttacagtatggaatgattgg

SEQ ID NO: 68 - DNA, 25 bp, Artificial Sequence
  probe
ccattattaaagcagctttagaacc

SEQ ID NO: 69 - DNA, 25 bp, Artificial Sequence
  probe
aagatagcgtttcagtttctgatgc

SEQ ID NO: 70 - DNA, 25 bp, Artificial Sequence
  probe
cctggaagctgtataatagattgta

SEQ ID NO: 71 - DNA, 25 bp, Artificial Sequence
  probe
atcccagaaggaaacggaaacttta

SEQ ID NO: 72 - DNA, 25 bp, Artificial Sequence
  probe
attgcgaatatgtagcagagccgtt

SEQ ID NO: 73 - DNA, 25 bp, Artificial Sequence
  probe
tgttgactataatcaattacaggag

SEQ ID NO: 74 - DNA, 25 bp, Artificial Sequence
  probe
tgatatatcctgaaacattaaaatt

SEQ ID NO: 75 - DNA, 25 bp, Artificial Sequence
  probe
aagtcctctttcagcaggtcaggtg

SEQ ID NO: 76 - DNA, 25 bp, Artificial Sequence
  probe
ccgtaacattacaacctcaagcgca

SEQ ID NO: 77 - DNA, 25 bp, Artificial Sequence
  probe
tcagtatggatatctaggaatgcca

SEQ ID NO: 78 - DNA, 24 bp, Artificial Sequence
  probe
cagcacacaggacagggagccata

SEQ ID NO: 79 - DNA, 25 bp, Artificial Sequence
  probe
agtggaaagtgttacctcagggaat

SEQ ID NO: 80 - DNA, 25 bp, Artificial Sequence
  probe
cttaatagtccaactctttgtcaga

SEQ ID NO: 81 - DNA, 25 bp, Artificial Sequence
  probe
tttctgcaagcagaggttgccaatg

SEQ ID NO: 82 - DNA, 25 bp, Artificial Sequence
  probe
aggactggcaatagcatctgataag

SEQ ID NO: 83 - DNA, 25 bp, Artificial Sequence
  probe
ggcattcctacttatgccatgtcaa

SEQ ID NO: 84 - DNA, 25 bp, Artificial Sequence
  probe
tttgttctctatcttaagaggagac

SEQ ID NO: 85 - DNA, 25 bp, Artificial Sequence
  probe
tactgatcttgtggagtggtcattc

SEQ ID NO: 86 - DNA, 25 bp, Artificial Sequence
  probe
ttcctcacagtacagttaagacttt

SEQ ID NO: 87 - DNA, 25 bp, Artificial Sequence
  probe
tagttgtccctttaaccaaggaaca

SEQ ID NO: 88 - DNA, 25 bp, Artificial Sequence
  probe
gttagacaagcctttatcaattctg

SEQ ID NO: 89 - DNA, 25 bp, Artificial Sequence
  probe
aattgactacttggattctacctaa

SEQ ID NO: 90 - DNA, 25 bp, Artificial Sequence
  probe
attaccagacgtgaacctttagaaa

SEQ ID NO: 91 - DNA, 25 bp, Artificial Sequence
  probe
tcaatcggctcaaagagcagagttg

SEQ ID NO: 92 - DNA, 25 bp, Artificial Sequence
  probe
ttgcagtcattacagtgttacaaga

SEQ ID NO: 93 - DNA, 25 bp, Artificial Sequence
  probe
tcggattctgcatatgtagtacagg

SEQ ID NO: 94 - DNA, 25 bp, Artificial Sequence
  probe
tacaagggatgttgagacagctcta

SEQ ID NO: 95 - DNA, 25 bp, Artificial Sequence
  probe
attgtacaacattgcacccagtgtc

SEQ ID NO: 96 - DNA, 25 bp, Artificial Sequence
  probe
agtcttagacctgcccactcaagag

SEQ ID NO: 97 - DNA, 25 bp, Artificial Sequence
  probe
tatggcaaatggatgtcacacatgt

SEQ ID NO: 98 - DNA, 26 bp, Artificial Sequence
  probe
ccttcatttgggaagattatcatatg

SEQ ID NO: 99 - DNA, 25 bp, Artificial Sequence
  probe
ttcacatttcatgtgtgcaacttgc

SEQ ID NO: 100 - DNA, 25 bp, Artificial Sequence
  probe
aaacaggagaaagtacttcccatgt

SEQ ID NO: 101 - DNA, 25 bp, Artificial Sequence
  probe
cacatacaacaggaattccttataa

SEQ ID NO: 102 - DNA, 25 bp, Artificial Sequence
  probe
tcccaaggacaggccatagttgaaa

SEQ ID NO: 103 - DNA, 25 bp, Artificial Sequence
  probe
gacagtaaggagtgtaccactcctc

SEQ ID NO: 104 - DNA, 25 bp, Artificial Sequence
  probe
gatgcaacttaatctagcactctat

SEQ ID NO: 105 - DNA, 25 bp, Artificial Sequence
  probe
tttccattgggtatcattatcctcc

SEQ ID NO: 106 - DNA, 25 bp, Artificial Sequence
  probe
atttgcctagggagagcaccaggat

SEQ ID NO: 107 - DNA, 25 bp, Artificial Sequence
  probe
tagaagtacctactgtcagtcctaa

SEQ ID NO: 108 - DNA, 25 bp, Artificial Sequence
  probe
agtagattcacttatcacatggtaa

SEQ ID NO: 109 - DNA, 25 bp, Artificial Sequence
  probe
attcctaaaggatcaaagaatacag

SEQ ID NO: 110 - DNA, 25 bp, Artificial Sequence
  probe
agttttagtttgggaagaatgtgtg

SEQ ID NO: 111 - DNA, 25 bp, Artificial Sequence
  probe
agattgggcacctcgaggtcaattc

SEQ ID NO: 112 - DNA, 25 bp, Artificial Sequence
  probe
accacaattgctcaggacaaactca

SEQ ID NO: 113 - DNA, 25 bp, Artificial Sequence
  probe
gaacatccagaattgtggaggctta

SEQ ID NO: 114 - DNA, 25 bp, Artificial Sequence
  probe
tgtggcctcacaccacattagaatt

SEQ ID NO: 115 - DNA, 25 bp, Artificial Sequence
  probe
ttcctttacaaagttgcgtaaagcc

SEQ ID NO: 116 - DNA, 25 bp, Artificial Sequence
  probe
ccttatatgctagttgtaggaaata

SEQ ID NO: 117 - DNA, 25 bp, Artificial Sequence
  probe
ccgtattctgctggtgagagcaaga

SEQ ID NO: 118 - DNA, 25 bp, Artificial Sequence
  probe
aaggcatgtggatccctgtgtccac

SEQ ID NO: 119 - DNA, 25 bp, Artificial Sequence
  probe
actttaattgcagtgattatgggat

SEQ ID NO: 120 - DNA, 25 bp, Artificial Sequence
  probe
aattgcagtcacagctacggctgct

SEQ ID NO: 121 - DNA, 25 bp, Artificial Sequence
  probe
gatcttagacaaactgtcatttgga

SEQ ID NO: 122 - DNA, 25 bp, Artificial Sequence
  probe
gggagacaggctcatgaccttagaa

SEQ ID NO: 123 - DNA, 25 bp, Artificial Sequence
  probe
gtctgagcatcactgggacatggtt

SEQ ID NO: 124 - DNA, 25 bp, Artificial Sequence
  probe
gacgccatctacagggaagagaaga

SEQ ID NO: 125 - DNA, 25 bp, Artificial Sequence
  probe
ttagtctgcaggtgtacccaacagc

SEQ ID NO: 126 - DNA, 25 bp, Artificial Sequence
  probe
ccgaagagacagtgacatcgagaac

SEQ ID NO: 127 - DNA, 25 bp, Artificial Sequence
  probe
tcagattgttactgtgtctgtatag

SEQ ID NO: 128 - DNA, 25 bp, Artificial Sequence
  probe
aagaagtagacataggagactccat

SEQ ID NO: 129 - DNA, 25 bp, Artificial Sequence
  probe
gtgctctctgaaacatgtgctgtgt

SEQ ID NO: 130 - DNA, 25 bp, Artificial Sequence
  probe
aaactcagggttaaatggattaagg

SEQ ID NO: 131 - DNA, 25 bp, Artificial Sequence
  probe
acagatgcttgaaggcagcatgctc

SEQ ID NO: 132 - DNA, 25 bp, Artificial Sequence
  probe
ttaagagtcatcaccactccctaat

SEQ ID NO: 133 - DNA, 25 bp, Artificial Sequence
  probe
ctgtgctgaggaggattagtataag

SEQ ID NO: 134 - DNA, 25 bp, Artificial Sequence
  probe
ggaaagcatgcctcttgcagttgag

SEQ ID NO: 135 - DNA, 25 bp, Artificial Sequence
  probe
cgattgtacgttccacctactgaga

SEQ ID NO: 136 - DNA, 25 bp, Artificial Sequence
  probe
agggagaaaccaccttagggctgga

SEQ ID NO: 137 - DNA, 25 bp, Artificial Sequence
  probe
tcctttaccttgtctatgatgcaaa

SEQ ID NO: 138 - DNA, 25 bp, Artificial Sequence
  probe
acctttgttcacgtgtttgtctgct

SEQ ID NO: 139 - DNA, 25 bp, Artificial Sequence
  probe
ttagtataagaggaaagcatgcctc

SEQ ID NO: 140 - DNA, 25 bp, Artificial Sequence
  probe
tgcagttgagagaagaggaagacat

SEQ ID NO: 141 - DNA, 25 bp, Artificial Sequence
  probe
gtgggcagcaatactgcttcgtaaa

SEQ ID NO: 142 - DNA, 25 bp, Artificial Sequence
  probe
cattgagatgtttatgtgtatgcat

SEQ ID NO: 143 - DNA, 25 bp, Artificial Sequence
  probe
taccttgtctatgatgcaaacacct

SEQ ID NO: 144 - DNA, 25 bp, Artificial Sequence
  probe
tgttcacgtgtttgtctgctgaccc

SEQ ID NO: 145 - DNA, 25 bp, Artificial Sequence
  probe
tctcggagaaacacccacgaatgat

SEQ ID NO: 146 - DNA, 25 bp, Artificial Sequence
  probe
aataaatactaagggaactcagagg

SEQ ID NO: 147 - DNA, 25 bp, Artificial Sequence
  probe
tctcattccaccttatgagaaacac

SEQ ID NO: 148 - DNA, 25 bp, Artificial Sequence
  probe
cacaggtgtggaggggcaacccacc

SEQ ID NO: 149 - DNA, 318 bp, Homo sapiens
atgaacccatcagagatgcaaagaaaagcacctccgcggagacggagacaccgcaatcgagcaccgttgactcacaagatgaacaaaatggtgacgtcagaagaacagatgaagttgccatccaccaagaaggcagagccgccgacttgggcacaactaaagaagctgacgcagttagctacaaaatatctagagaacacaaaggtgacacaaaccccagagagtatgctgcttgcagccttgatgattgtatcaatggtgtctgcaggtgtacccaacagctccgaagagacagcgaccatcgagaacgggccatga

SEQ ID NO: 150 - DNA, 9472 bp, Homo sapiens
tgtggggaaaagcaagagagatcagattgttactgtgtctgtgtagaaagaagtagacataggagactccattttgttatgtactaagaaaaattcttctgccttgagattctgttaatctatgaccttacccccaaccccgtgctctctgaaacatgtgctgtgtcaactcagagttaaatggattaagggcggtgcaggatgtgctttgttaaacagatgcttgaaggcagcatgctccttaagagtcatcaccactccctaatctcaagtacccagggacacaaaaactgcggaaggccgcagggacctctgcctaggaaagccaggtattgtccaaggtttctccccatgtgatagtctgaaatatggcctcgtgggaagggaaagacctgaccgtcccccagcccgacacccgtaaagggtctgtgctgaggaggattagtaaaagaggaaggaatgcctcttgcagttgagacaagaggaaggcatctgtctcctgcctgtccctgggcaatggaatgtctcggtataaaacccgattgtatgctccatctactgagatagggaaaaaccgccttagggctggaggtgggacctgcgggcagcaatactgctttgtaaagcactgagatgtttatgtgtatgcatatctaaaagcacagcacttaatcctttacattgtctatgatgcaaagacctttgttcacgtgtttgtctgctgaccctctccccacaattgtcttgtgaccctgacacatccccctctttgagaaacacccacagatgatcaataaatactaagggaactcagaggctggcgggatcctccatatgctgaacgctggttccccgggtccccttatttctttctctatactttgtctctgtgtctttttcttttccaaatctctcgtcccaccttacgagaaacacccacaggtgtgtaggggcaacccacccctacatctggtgcccaacgtggaggcttttctctagggtgaaggtacgctcgagcgtggtcattgaggacaagtcgacgagagatcccgagtacgtctacagtcagccttacggtaagcttgtgcgctcggaagaagctagggtgataatggggcaaactaaaagtaaaattaaaagtaaatatgcctcttatctcagctttattaaaattcttttaaaaagagggggagttaaagtatctacaaaaaatctaatcaagctatttcaaataatagaacaattttgcccatggtttccagaacaaggaactttagatctaaaagattggaaaagaattggtaaggaactaaaacaagcaggtaggaagggtaatatcattccacttacagtatggaatgattgggccattattaaagcagctttagaaccatttcaaacagaagaagatagcgtttcagtttctgatgcccctggaagctgtataatagattgtaatgaaaacacaaggaaaaaatcccagaaagaaacggaaggtttacattgcgaatatgtagcagagccggtaatggctcagtcaacgcaaaatgttgactataatcaattacaggaggtgatatatcctgaaacgttaaaattagaaggaaaaggtccagaattagtggggccatcagagtctaaaccacgaggcacaagtcctcttccagcaggtcaggtgcccgtaacattacaacctcaaaagcaggttaaagaaaataagacccaaccgccagtagcctatcaatactggccgccggctgaacttcagtatcggccacccccagaaagtcagtatggatatccaggaatgcccccagcaccacagggcagggcgccataccctcagccgcccactaggagacttaatcctacggcaccacctagtagacagggtagtgaattacatgaaattattgataaatcaagaaaggaaggagatactgaggcatggcaattcccagtaacgttagaaccgatgccacctggagaaggagcccaagagggagagcctcccacagttgaggccagatacaagtctttttcgataaaaatgctaaaagatatgaaagagggagtaaaacagtatggacccaactccccttatatgaggacattattagattccattgctcatggacatagactcattccttatgattgggagattctggcaaaatcgtctctctcaccctctcaatttttacaatttaagacttggtggattgatggggtacaagaacaggtccgaagaaatagggctgccaatcctccagttaacatagatgcagatcaactattaggaataggtcaaaattggagtactattagtcaacaagcattaatgcaaaatgaggccattgagcaagttagagctatctgccttagagcctgggaaaaaatccaagacccaggaagtacctgcccctcatttaatacagtaagacaaggttcaaaagagccctatcctgattttgtggcaaggctccaagatgttgctcaaaagtcaattgccgatgaaaaagcccgtaaggtcatagtggagttgatggcatatgaaaacgccaatcctgagtgtcaatcagccattaagccattaaaaggaaaggttcctgcaggatcagatgtaatctcagaatatgtaaaagcctgtgatggaatcggaggagctatgcataaagctatgcttatggctcaagcaataacaggagttgttttaggaggacaagttagaacatttggaggaaaatgttataattgtggtcaaattggtcacttaaaaaagaattgcccagtcttaaacaaacagaatataactattcaagcaactacaacaggtagagagccacctgacttatgtccaagatgtaaaaaaggaaaacattgggctagtcaatgtcgttctaaatttgataaaaatgggcaaccattgtcgggaaacgagcaaaggggccagcctcaggccccacaacaaactggggcattcccaattcagccatttgttcctcagggttttcagggacaacaacccccactgtcccaagtgtttcagggaataagccagttaccacaatacaacaattgtcccccgccacaagcggcagtgcagcagtagatttatgtactatacaagcagtctctctgcttccaggggagcccccacaaaaaatccccacaggggtatatggccccctgcctgaggggactgtaggactaatcttgggaagatcaagtctaaatctaaaaggagttcaaattcatactagtgtggttgattcagactataaaggcgaaattcaattggttattagctcttcaattccttggagtgccagtccaggagacaggattgctcaattattactcctgccatatattaagggtggaaatagtgaaataaaaagaataggagggcttggaagcactgatccaacaggaaaggctgcatattgggcaagtcaggtctcagagaacagacctgtgtgtaaggccattattcaaggaaaacagtttgaagggttggtagacactggagcagatgtctctatcattgctttaaatcagtggccaaaaaattggcctaaacaaaaggctgttacaggacttgtcggcataggcacagcctcagaagtgtatcaaagtacggagattttacattgcttagggccagataatcaagaaagtactgttcagccaatgattacttcaattcctcttaatctgtggggtcgagatttattacaacaatggggtgcggaaatcaccatgcccgctccattatatagccccacgagtcaaaaaatcatgaccaagatgggatatataccaggaaagggactagggaaaaatgaagatggcattaaaattccagttgaggctaaaataaatcaaaaaagagaaggaatagggtatcctttttaggggcggccactgtagagcctcctaaacccataccattaacttggaaaacagaaaaaccggtgtgggtaaatcagtggccgctaccaaaacaaaaactggaggctttacatttattagcaaatgaacagttagaaaagggtcatattgagccttcgttctcaccttggaattctcctgtgtttgtaattcagaagaaatcaggcaaatggcgtatgttaactgacttaagggctgtaaacgccgtaattcaacccatggggcctctccaacccgggttgccctctccggccatgatcccaaaagattggcctttaattataattgatctaaaggattgcttttttaccatccctctggcagagcaggattgtgaaaaatttgcctttactataccagccataaataataaagaaccagccaccaggtttcagtggaaagtgttacctcagggaatgcttaatagtccaactatttgtcagacttttgtaggtcgagctcttcaaccagttagagaaaagttttcagactgttatattattcattatattgatgatattttatgtgctgcagaaacgaaagataaattaattgactgttatacatttctgcaagcagaggttgccaatgctggactggcaatagcatctgataagatccaaacctctactccttttcattatttagggatgcagatagaaaatagaaaaattaagccacaaaaaatagaaataagaaaagacacattaaaaacactaaatgattttcaaaaattactaggagatattaattggattcggccaactctaggcattcctacttatgccatgtcaaatttgttctctatcttaagaggagactcagacttaaatagtaaaagaatgttaaccccagaggcaacaaaagaaattaaattagtggaagaaaaaattcagtcagcgcaaataaatagaatagatcccttagccccactccaacttttgatttttgccactgcacattctccaacaggcatcattattcaaaatactgatcttgtggagtggtcattccttcctcacagtacagttaagacttttacattgtacttggatcaaatagctacattaatcggtcagacaagattacgaataataaaattatgtggaaatgacccagacaaaatagttgtccctttaaccaaggaacaagttagacaagcctttatcaattctggtgcatggcagattggtcttgctaattttgtgggaattattgataatcattacccaaaaacaaagatcttccagttcttaaaattgactacttggattctacctaaaattaccagacgtgaacctttagaaaatgctctaacagtatttactgatggttccagcaatggaaaagcagcttacacagggccgaaagaacgagtaatcaaaactccatatcaatcggctcaaagagcagagttggttgcagtcattacagtgttacaagattttgaccaacctatcaatattatatcagattctgcatatgtagtacaggctacaagggatgttgagacagctctaattaaatatagcatggatgatcagttaaaccagctattcaatttattacaacaaactgtaagaaaaagaaatttcccattttatattactcatattcgagcacacactaatttaccagggcctttgactaaagcaaatgaacaagctgacttactggtatcatctgcactcataaaagcacaagaacttcatgctttgactcatgtaaatgcagcaggattaaaaaacaaatttgatgtcacatggaaacaggcaaaagatattgtacaacattgcacccagtgtcaagtcttacacctgcccactcaagaggcaggagttaatcccagaggtctgtgtcctaatgcattatggcaaatggatgtcacgcatgtaccttcatttggaagattatcatatgttcatgtaacagttgatacttattcacatttcatatgggcaacttgccaaacaggagaaagtacttcccatgttaaaaaacatttattgtcttgttttgctgtaatgggagttccagaaaaaatcaaaactgacaatggaccaggatattgtagtaaagctttccaaaaattcttaagtcagtggaaaatttcacatacaacaggaattccttataattcccaaggacaggccatagttgaaagaactaatagaacactcaaaactcaattagttaaacaaaaagaagggggagacagtaaggagtgtaccactcctcagatgcaacttaatctagcactctatactttaaattttttaaacatttatagaaatcagactactacttctgcagaacaacatcttactggtaaaaagaacagcccacatgaaggaaaactaatttggtggaaagataataaaaataagacatgggaaatagggaaggtgataacgtgggggagaggttttgcttgtgtttcaccaggagaaaatcagcttcctgtttggatacccactagacatttgaagttctacaatgaacccatcagagatgcaaagaaaagcacctccgcggagacggagacaccgcaatcgagcaccgttgactcacaagatgaacaaaatggtgacgtcagaagaacagatgaagttgccatccaccaagaaggcagagccgccgacttgggcacaactaaagaagctgacgcagttagctacaaaatatctagagaacacaaaggtgacacaaaccccagagagtatgctgcttgcagccttgatgattgtatcaatggtggtaagtctccctatgcctgcaggagcagctgcagctaactatacctactgggcctatgtgcctttcccgcccttaattcgggcagtcacatggatggataatcctatagaagtatatgttaatgatagtgtatgggtacctggccccatagatgatcgctgccctgccaaacctgaggaagaagggatgatgataaatatttccattgggtatcgttatcctcctatttgcctagggagagcaccaggatgtttaatgcctgcagtccaaaattggttggtagaagtacctactgtcagtcccatcagtagattcacttatcacatggtaagcgggatgtcactcaggccacgggtaaattatttacaagacttttcttatcaaagatcattaaaatttagacctaaagggaaaccttgccccaaggaaattcccaaagaatcaaaaaatacagaagttttagtttgggaagaatgtgtggccaatagtgcggtgatattacaaaacaatgaatttggaactattatagattgggcacctcgaggtcaattctaccacaattgctcaggacaaactcagtcgtgtccaagtgcacaagtgagtccagctgttgatagcgacttaacagaaagtttagacaaacataagcataaaaaattgcagtctttctacccttgggaatggggagaaaaaggaatctctaccccaagaccaaaaataataagtcctgtttctggtcctgaacatccagaattatggaggcttactgtggcctcacaccacattagaatttggtctggaaatcaaactttagaaacaagagatcgtaagccattttatactgtcgacctaaattccagtctaacagttcctttacaaagttgcgtaaagcccccttatatgctagttgtaggaaatatagttattaaaccagactcccagactataacctgtgaaaattgtagattgcttacttgcattgattcaacttttaattggcaacaccgtattctgctggtgagagcaagagagggcgtgtggatccctgtgtccatggaccgaccgtgggaggcctcaccatccatccatattttgactgaagtattaaaaggtgttttaaatagatccaaaagattcatttttactttaattgcagtgattatgggattaattgcagtcacagctacggctgctgtagcaggagttgcattgcactcttctgttcagtcagtaaactttgttaatgattggcaaaaaaattctacaagattgtggaattcacaatctagtattgatcaaaaattggcaaatcaaattaatgatcttagacaaactgtcatttggatgggagacagactcatgagcttagaacatcgtttccagttacaatgtgactggaatacgtcagatttttgtattacaccccaaatttataatgagtctgagcatcactgggacatggttagacgccatctacagggaagagaagataatctcactttagacatttccaaattaaaagaacaaattttcgaagcatcaaaagcccatttaaatttggtgccaggaactgaggcaattgcaggagttgctgatggcctcgcaaatcttaaccctgtcacttgggttaagaccattggaagtactacgattataaatctcatattaatccttgtgtgcctgttttgtctgttgttagtctgcaggtgtacccaacagctccgaagagacagcgaccatcgagaacgggccatgatgacgatggcggttttgtcgaaaagaaaagggggaaatgtggggaaaagcaagagagatcagattgttactgtgtctgtgtagaaagaagtagacataggagactccattttgttatgtactaagaaaaattcttctgccttgagattctgttaatctatgaccttacccccaaccccgtgctctctgaaacatgtgctgtgtcaactcagagttgaatggattaagggcggtgcaggatgtgctttgttaaacagatgcttgaaggcagcatgctccttaagagtcatcaccactccctaatctcaagtacccagggacacaaaaactgcggaaggccgcagggacctctgcctaggaaagccaggtattgtccaaggtttctccccatgtgatagtctgaaatatggcctcgtgggaagggaaagacctgaccgtcccccagcccgacacccgtaaagggtctgtgctgaggaggattagtaaaagaggaaggaatgcctcttgcagttgagacaagaggaaggcatctgtctcctgcctgtccctgggcaatggaatgtctcggtataaaacccgattgtatgctccatctactgagatagggaaaaaccgccttagggctggaggtgggacctgcgggcagcaatactgctttgtaaagcattgagatgtttatgtgtatgcatatctaaaagcacagcacttaatcctttacattgtctatgatgcaaagacctttgttcacgtgtttgtctgctgaccctctccccacaattgtcttgtgaccctgacacatccccctctttgagaaacacccacagatgatcaataaatactaagggaactcagaggctggcgggatcctccatatgctgaacgctggttccccgggtccccttatttctttctctatactttgtctctgtgtctttttcttttccaaatctctcgtcccaccttacgagaaacacccacaggtgtgtaggggcaacccacccctaca

SEQ ID NO: 151 - protein, 356 aa, Artificial Sequence
  MMTV antigen
ESYWAYLPKPPILHPVGWGSTDPIRVLTNQTMYLGGSPDFHGFRNMSGNVHFEGKSDTLPICFSFSFSTPTGCFQVDKQVFLSDTPTVDNNKPGGKGDKRRMWELWLHTLGNSGANTKLVPIKKKLPPKYPHCQIAFKKDAFWEGDESAPPRWLPCAFPDKGVSFSPKGALGLLWDFSLPSPSVDQSDQIKSKKDLFGNYTPPVNKEVHRWYEAGWVEPTWFWENSPKDPNDRDFTALVPHTELFRLVAASRHLILKRPGFQEHEMIPTSACVTYPYAILLGLPQLIDIEKRGSTFHISCSSCRLTNCLDSSAYDYAAIIVKRPPYVLLPVDIGDEPWFDDSAIQTFRYATDLIRA

SEQ ID NO: 152 - DNA, 2414 bp, Artificial Sequence
  GFP Reporter
gaacaaacgacccaacacccgtgcgttttattctgtctttttattgccgatcccctcagaagaactcgtcaagaaggcgatagaaggcgatgcgctgcgaatcgggagcggcgataccgtaaagcacgaggaagcggtcagcccattcgccgccaagctcttcagcaatatcacgggtagccaacgctatgtcctgatagcggtcggccgctttacttgtacagctcgtccatgccgagagtgatcccggcggcggtcacgaactccagcaggaccatgtgatcgcgcttctcgttggggtctttgctcagggcggactgggtgctcaggtagtggttgtcgggcagcagcacggggccgtcgccgatgggggtgttctgctggtagtggtcggccaggtgagtccaggagatgtttcagcactgttgcctttagtctcgaggcaacttagacaactgagtattgatctgagcacagcagggtgtgagctgtttgaagatactggggttgggggtgaagaaactgcagaggactaactgggctgagacccagtggcaatgttttagggcctaaggaatgcctctgaaaatctagatggacaactttgactttgagaaaagagaggtggaaatgaggaaaatgacttttctttattagatttcggtagaaagaactttcatctttcccctatttttgttattcgttttaaaacatctatctggaggcaggacaagtatggtcattaaaaagatgcaggcagaaggcatatattggctcagtcaaagtggggaactttggtggccaaacatacattgctaaggctattcctatatcagctggacacatataaaatgctgctaatgcttcattacaaacttatatcctttaattccagatgggggcaaagtatgtccaggggtgaggaacaattgaaacatttgggctggagtagattttgaaagtcagctctgtgtgtgtgtgtgtgtgtgtgtgtgtgtgtgtgtgcgcgcacgtgtgtttgtgtgtgtgtgagagcgtgtgtttcttttaacgttttcagcctacagcatacagggttcatggtggcaagaagataacaagatttaaattatggccagtgactagtgctgcaagaagaacaactacctgcatttaatgggaaagcaaaatctcaggctttgagggaagttaacataggcttgattctgggtggaagctgggtgtgtagttatctggaggccaggctggagctctcagctcactatgggttcatctttattgtctcctttcatctcaacagctgcacgctgccgtcctcgatgttgtggcggatcttgaagttcaccttgatgccgttcttctgcttgtcggccatgatatagacgttgtggctgttgtagttgtactccagcttgtgccccaggatgttgccgtcctccttgaagtcgatgcccttcagctcgatgcggttcaccagggtgtcgccctcgaacttcacctcggcgcgggtcttgtagttgccgtcgtccttgaagaagatggtgcgctcctggacgtagccttcgggcatggcggacttgaagaagtcgtgctgcttcatgtggtcggggtagcggctgaagcactgcacgccgtaggtcagggtggtcacgagggtgggccagggcacgggcagcttgccggtggtgcagatgaacttcagggtcagcttgccgtaggtggcatcgccctcgccctcgccggacacgctgaacttgtggccgtttacgtcgccgtccagctcgaccaggatgggcaccaccccggtgaacagctcctcgcccttgctcaccatggtggcgaattcgaagcttgagctcgagatctgagtccggtagcgctagcggatctgacggttcactaaaccagctctgcttatatagacctcccaccgtacacgcctaccgcccatttgcgtcaatggggcggagttgttacgacattttggaaagtcccgttgattttggtgccaaaacaaactcccattgacgtcaatggggtggagacttggaaatccccgtgagtcaaaccgctatccacgcccattgatgtactgccaaaaccgcatcaccatggtaatagcgatgactaatacgtagatgtactgccaagtaggaaagtcccataaggtcatgtactgggcataatgccaggcgggccatttaccgtcattgacgtcaatagggggcgtacttggcatatgatacacttgatgtactgccaagtgggcagtttaccgtaaatactccacccattgacgtcaatggaaagtccctattggcgttactatgggaacatacgtcattattgacgtcaatgggcgggggtcgttgggcggtcagccaggcgggccatttaccgtaagttatgtaacg

SEQ ID NO: 153 - DNA, 808 bp, Artificial Sequence
  CMV-GFP
gcaaatgggcggtaggcgtgtacggtgggaggtctatataagcagagctggtttagtgaaccgtcagatccgctagcgctaccggtcgccaccatggtgagcaagggcgaggagctgttcaccggggtggtgcccatcctggtcgagctggacggcgacgtaaacggccacaagttcagcgtgtccggcgagggcgagggcgatgccacctacggcaagctgaccctgaagttcatctgcaccaccggcagctgcccgtgccctggcccaccctcgtgaccaccctgacctacggcgtgcagtgcttcagccgctaccccgaccacatgaagcagcacgacttcttcaagtccgccatgcccgaaggctacgtccaggagcgcaccatcttcttcaaggacgacggcaactacaagacccgcgccgaggtgaagttcgaggcgacaccctggtgaaccgcatcgagctgaagggcatcgacttcaaggaggacggcaacatcctggggcacaagctggagtacaactacaacagccacaacgtctatatcatggccgacaagcagaagaacggcatcaaggtgaacttcaagatccgccacaacatcgaggacggcagcgtgcagctcgccgaccactaccagcagaacacccccatcggcgacggccccgtgctgctgcccgacaaccactacctgagcacccagtccgccctgagcaaagaccccaacgagaagcgcgatcacatggtcctgctggagttcgtgaccgccgccgggatcactctcggcatggacgagctgtacaag